European Patent Application EP 4 600 650 A2, published August 13, 2025. Title: IMPROVED METHODS AND COMPOSITIONS FOR SYNTHETIC BIOMARKERS. Applicant: EARLI INC. The sequence listing filed with the application follows.

SEQUENCE LISTING (7 sequences)

SEQ ID NO: 1 - DNA, 4098 bp, synthetic construct
  misc_feature 1..4098: note = Description of Artificial Sequence: Synthetic polynucleotide
  source 1..4098: mol_type = other DNA
ccccaactggggtaacctttgggctccccgggcgcgactagtaataaaatatctttattttcattacatctgtgtgttggttttttgtgtgaatcgatagtactaacatacgctctccatcaaaacaaaacgaaacaaaacaaactagcaaaataggctgtccccagtgcaagtgcaggtgccagaacatttctctactagtgccatagaaccagagaagtgagtggatgtgatgcccagctccagaagtgactccagaacaccctgttccaaagcagaggacacactgattttttttttaataggctgcaggacttactgttggtgggacgccctgctttgcgaagggaaaggaggagtttgccctgagcacaggcccccaccctccactgggctttccccagctcccttgtcttcttatcacggtagtggcccagtccctggcccctgactccagaaggtggccctcctggaaacccaggtcgtgcagtcaacgatgtactcgccgggacagcgatgtctgctgcactccatccctcccctgttcatttgtccttcatgcccgtctggagtagatgctttttgcagaggtggcaccctgtaaagctctcctgtctgactttttttttttttttagactgagttttgctcttgttgcctaggctggagtgcaatggcacaatctcagctcactgcaccctctgcctcccgggttcaagcgattctcctgcctcagcctcccgagtagttgggattacaggcatgcaccaccacgcccagctaatttttgtatttttagtagagacaaggtttcaccgtgatggccaggctggtcttgaactccaggactcaagtgatgctcctgcctaggcctctcaaagtgttgggattacaggcgtgagccactgcacccggcctgcacgcgttctttgaaagcagtcgagggggcgctaggtgtgggcagggacgagctggcgcggcgtcgctgggtgcaccgcgaccacgggcagagccacgcggcgggaggactacaactcccggcacaccccgcgccgccccgcctctactcccagaaggccgcggggggtggaccgcctaagagggcgtgcgctcccgacatgccccgcggcgcgccattaaccgccagatttgaatcgcgggacccgttggcagaggtgggaattcaccggtcaccatggttctggggccctgcatgctgctgctgctgctgctgctgggcctgaggctacagctctccctgggcatcatcccagttgaggaggagaacccggacttctggaaccgcgaggcagccgaggccctgggtgccgccaagaagctgcagcctgcacagacagccgccaagaacctcatcatcttcctgggcgatgggatgggggtgtctacggtgacagctgccaggatcctaaaagggcagaagaaggacaaactggggcctgagatacccctggctatggaccgcttcccatatgtggctctgtccaagacatacaatgtagacaaacatgtgccagacagtggagccacagccacggcctacctgtgcggggtcaagggcaacttccagaccattggcttgagtgcagccgcccgctttaaccagtgcaacacgacacgcggcaacgaggtcatctccgtgatgaatcgggccaagaaagcagggaagtcagtgggagtggtaaccaccacacgagtgcagcacgcctcgccagccggcacctacgcccacacggtgaaccgcaactggtactcggacgccgacgtgcctgcctcggcccgccaggaggggtgccaggacatcgctacgcagctcatctccaacatggacattgatgtgatcctgggtggaggccgaaagtacatgtttcgcatgggaaccccagaccctgagtacccagatgactacagccaaggtgggaccaggctggacgggaagaatctggtgcaggaatggctggcgaagcgccagggtgcccggtatgtgtggaaccgcactgagctcatgcaggcttccctggacccgtctgtgacccatctcatgggtctctttgagcctggagacatgaaatacgagatccaccgagactccacactggacccctccctgatggagatgacagaggctgccctgcgcctgctgagcaggaacccccgcggcttcttcctcttcgtggagggtggtcgcatcgaccacggtcatcacgaaagcagggcttaccgggcactgactgagacgatcatgttcgacgacgccattgagagggcgggccagctcaccagcgaggaggacacgctgagcctcgtcactgccgaccactcccacgtcttctccttcggaggctaccccctgcgagggagctccatcttcgggctggcccctggcaaggcccgggacaggaaggcctacacggtcctcctatacggaaacggtccaggctatgtgctcaaggacggcgcccggccggatgttaccgagagcgagagcgggagccccgagtatcggcagcagtcagcagtgcccctggacgaagagacccacgcaggcgaggacgtggcggtgttcgcgcgcggcccgcaggcgcacctggttcacggcgtgcaggagcagaccttcatagcgcacgtcatggccttcgccgcctgcctggagccctacaccgcctgcgacctggcgccccccgccggcaccaccgacgccgcgcacccggggcggtcccggtccaagcgtctggattgagctagcttcgaatttaaatcggatccctgcaggagctcgtcgacaatcaacctctggattacaaaatttgtgaaagattgactggtattcttaactatgttgctccttttacgctatgtggatacgctgctttaatgcctttgtatcatgctattgcttcccgtatggctttcattttctcctccttgtataaatcctggttgctgtctctttatgaggagttgtggcccgttgtcaggcaacgtggcgtggtgtgcactgtgtttgctgacgcaacccccactggttggggcattgccaccacctgtcagctcctttccgggactttcgctttccccctccctattgccacggcggaactcatcgccgcctgccttgcccgctgctggacaggggctcggctgttgggcactgacaattccgtggtgttgtcggggaaatcatcgtcctttccttggctgctcgcctgtgttgccacctggattctgcgcgggacgtccttctgctacgtcccttcggccctcaatccagcggaccttccttcccgcggcctgctgccggctctgcggcctcttccgcgtcttcgccttcgccctcagacgagtcggatctccctttgggccgcctccccgcctggtacctttaagaccaatgacttacaaggcagctgtagatcttagccactttttaaaagaaaaggggggactggaagggctaattcactcccaacgaaaataagatctgctttttgcttgtactgggtctctctggttagaccagatctgagcctgggagctctctggctaactagggaacccactgcttaagcctcaataaagcttgccttgagtgcttcaagtagtgtgtgcccgtctgttgtgtgactctggtaactagagatccctcagacccttttagtcagtgtggaaaatctctagcagtagtagttcatgtcatcttattattcagtatttataacttgcaaagaaatgaatatcagagagtgagaggaacttgtttattgcagcttataatggttacaaataaagcaatagcatcacaaatttcacaaataaagcatttttttcactgcattctagttgtggtttgtccaaactcatcaatgtatcttatcatgtctggctctagctatcccgcccctaactccgcccagttccgcccattctccgcccctcccgcccctaactccgcccaatggctgactaattttttttatttatgcagaggccgaggccgcctcggcctctgagctattccagaagtagtgaggaggcttttttggaggcctagacttttgcagatcgacccatgggggcccg

SEQ ID NO: 2 - DNA, 4256 bp, synthetic construct
  misc_feature 1..4256: note = Description of Artificial Sequence: Synthetic polynucleotide
  source 1..4256: mol_type = other DNA
ccccaactggggtaacctttgggctccccgggcgcgactagtaataaaatatctttattttcattacatctgtgtgttggttttttgtgtgaatcgatagtactaacatacgctctccatcaaaacaaaacgaaacaaaacaaactagcaaaataggctgtccccagtgcaagtgcaggtgccagaacatttctctactagtgaattgatgccatagaaccagagaagtgagtggatgtgatgcccagctccagaagtgactccagaacaccctgttccaaagcagaggacacactgattttttttttaataggctgcaggacttactgttggtgggacgccctgctttgcgaagggaaaggaggagtttgccctgagcacaggcccccaccctccactgggctttccccagctcccttgtcttcttatcacggtagtggcccagtccctggcccctgactccagaaggtggccctcctggaaacccaggtcgtgcagtcaacgatgtactcgccgggacagcgatgtctgctgcactccatccctcccctgttcatttgtccttcatgcccgtctggagtagatgctttttgcagaggtggcaccctgtaaagctctcctgtctgactttttttttttttttagactgagttttgctcttgttgcctaggctggagtgcaatggcacaatctcagctcactgcaccctctgcctcccgggttcaagcgattctcctgcctcagcctcccgagtagttgggattacaggcatgcaccaccacgcccagctaatttttgtatttttagtagagacaaggtttcaccgtgatggccaggctggtcttgaactccaggactcaagtgatgctcctgcctaggcctctcaaagtgttgggattacaggcgtgagccactgcacccggcctgcacgcgttctttgaaagcagtcgagggggcgctaggtgtgggcagggacgagctggcgcggcgtcgctgggtgcaccgcgaccacgggcagagccacgcggcgggaggactacaactcccggcacaccccgcgccgccccgcctctactcccagaaggccgcggggggtggaccgcctaagagggcgtgcgctcccgacatgccccgcggcgcgccattaaccgccagatttgaatcgcgggacccgttggcagaggtggaagcttggcaatccggtactgttggtaaagccaccatggaagatgccaaaaacattaagaagggcccagcgccattctacccactcgaagacgggaccgccggcgagcagctgcacaaagccatgaagcgctacgccctggtgcccggcaccatcgcctttaccgacgcacatatcgaggtggacattacctacgccgagtacttcgagatgagcgttcggctggcagaagctatgaagcgctatgggctgaatacaaaccatcggatcgtggtgtgcagcgagaatagcttgcagttcttcatgcccgtgttgggtgccctgttcatcggtgtggctgtggccccagctaacgacatctacaacgagcgcgagctgctgaacagcatgggcatcagccagcccaccgtcgtattcgtgagcaagaaagggctgcaaaagatcctcaacgtgcaaaagaagctaccgatcatacaaaagatcatcatcatggatagcaagaccgactaccagggcttccaaagcatgtacaccttcgtgacttcccatttgccacccggcttcaacgagtacgacttcgtgcccgagagcttcgaccgggacaaaaccatcgccctgatcatgaacagtagtggcagtaccggattgcccaagggcgtagccctaccgcaccgcaccgcttgtgtccgattcagtcatgcccgcgaccccatcttcggcaaccagatcatccccgacaccgctatcctcagcgtggtgccatttcaccacggcttcggcatgttcaccacgctgggctacttgatctgcggctttcgggtcgtgctcatgtaccgcttcgaggaggagctattcttgcgcagcttgcaagactataagattcaatctgccctgctggtgcccacactatttagcttcttcgctaagagcactctcatcgacaagtacgacctaagcaacttgcacgagatcgccagcggcggggcgccgctcagcaaggaggtaggtgaggccgtggccaaacgcttccacctaccaggcatccgccagggctacggcctgacagaaacaaccagcgccattctgatcacccccgaaggggacgacaagcctggcgcagtaggcaaggtggtgcccttcttcgaggctaaggtggtggacttggacaccggtaagacactgggtgtgaaccagcgcggcgagctgtgcgtccgtggccccatgatcatgagcggctacgttaacaaccccgaggctacaaacgctctcatcgacaaggacggctggctgcacagcggcgacatcgcctactgggacgaggacgagcacttcttcatcgtggaccggctgaagagcctgatcaaatacaagggctaccaggtagccccagccgaactggagagcatcctgctgcaacaccccaacatcttcgacgccggggtcgccggcctgcccgacgacgatgccggcgagctgcccgccgcagtcgtcgtgctggaacacggtaaaaccatgaccgagaaggagatcgtggactatgtggccagccaggttacaaccgccaagaagctgcgcggtggtgttgtgttcgtggacgaggtgcctaaaggactgaccggcaagttggacgcccgcaagatccgcgagattctcattaaggccaagaagggcggcaagatcgccgtgtaatctagagctagcgaattcagatctgatatctctagagtcgagctagcttcgaatttaaatcggatccctgcaggagctcgtcgacaatcaacctctggattacaaaatttgtgaaagattgactggtattcttaactatgttgctccttttacgctatgtggatacgctgctttaatgcctttgtatcatgctattgcttcccgtatggctttcattttctcctccttgtataaatcctggttgctgtctctttatgaggagttgtggcccgttgtcaggcaacgtggcgtggtgtgcactgtgtttgctgacgcaacccccactggttggggcattgccaccacctgtcagctcctttccgggactttcgctttccccctccctattgccacggcggaactcatcgccgcctgccttgcccgctgctggacaggggctcggctgttgggcactgacaattccgtggtgttgtcggggaaatcatcgtcctttccttggctgctcgcctgtgttgccacctggattctgcgcgggacgtccttctgctacgtcccttcggccctcaatccagcggaccttccttcccgcggcctgctgccggctctgcggcctcttccgcgtcttcgccttcgccctcagacgagtcggatctccctttgggccgcctccccgcctggtacctttaagaccaatgacttacaaggcagctgtagatcttagccactttttaaaagaaaaggggggactggaagggctaattcactcccaacgaaaataagatctgctttttgcttgtactgggtctctctggttagaccagatctgagcctgggagctctctggctaactagggaacccactgcttaagcctcaataaagcttgccttgagtgcttcaagtagtgtgtgcccgtctgttgtgtgactctggtaactagagatccctcagacccttttagtcagtgtggaaaatctctagcagtagtagttcatgtcatcttattattcagtatttataacttgcaaagaaatgaatatcagagagtgagaggaacttgtttattgcagcttataatggttacaaataaagcaatagcatcacaaatttcacaaataaagcatttttttcactgcattctagttgtggtttgtccaaactcatcaatgtatcttatcatgtctggctctagctatcccgcccctaactccgcccagttccgcccattctccgcccctcccgcccctaactccgcccaatggctgactaattttttttatttatgcagaggccgaggccgcctcggcctctgagctattccagaagtagtgaggaggcttttttggaggcctagacttttgcagatcgacccatgggggcccg

SEQ ID NO: 3 - DNA, 281 bp, synthetic construct
  misc_feature 1..281: note = Description of Artificial Sequence: Synthetic polynucleotide
  source 1..281: mol_type = other DNA
ggcttgttgtccacaaccgttaaaccttaaaagctttaaaagccttatatattcttttttttcttataaaacttaaaaccttagaggctatttaagttgctgatttatattaattttattgttcaaacatgagagcttagtacgtgaaacatgagagcttagtacgttagccatgagagcttagtacgttagccatgagggtttagttcgttaaacatgagagcttagtacgttaaacatgagagcttagtacgtactatcaacaggttgaactgctgatc

SEQ ID NO: 4 - DNA, 139 bp, synthetic construct
  misc_feature 1..139: note = Description of Artificial Sequence: Synthetic polynucleotide
  source 1..139: mol_type = other DNA
gtagaattggtaaagagagtcgtgtaaaatatcgagttcgcacatcttgttgtctgattattgatttttggcgaaaccatttgatcatatgacaagatgtgtatctaccttaacttaatgattttgataaaaatcatta

SEQ ID NO: 5 - DNA, 3962 bp, synthetic construct
  misc_feature 1..3962: note = Description of Artificial Sequence: Synthetic polynucleotide
  source 1..3962: mol_type = other DNA
gccatagaaccagagaagtgagtggatgtgatgcccagctccagaagtgactccagaacaccctgttccaaagcagaggacacactgatttttttttttaataggctgcaggacttactgttggtgggacgccctgctttgcgaagggaaaggaggagtttgccctgagcacaggcccccaccctccactgggctttccccagctcccttgtcttcttatcacggtagtggcccagtccctggcccctgactccagaaggtggccctcctggaaacccaggtcgtgcagtcaacgatgtactcgccgggacagcgatgtctgctgcactccatccctcccctgttcatttgtccttcatgcccgtctggagtagatgctttttgcagaggtggcaccctgtaaagctctcctgtctgactttttttttttttttagactgagttttgctcttgttgcctaggctggagtgcaatggcacaatctcagctcactgcaccctctgcctcccgggttcaagcgattctcctgcctcagcctcccgagtagttgggattacaggcatgcaccaccacgcccagctaatttttgtatttttagtagagacaaggtttcaccgtgatggccaggctggtcttgaactccaggactcaagtgatgctcctgcctaggcctctcaaagtgttgggattacaggcgtgagccactgcacccggcctgcacgcgttctttgaaagcagtcgagggggcgctaggtgtgggcagggacgagctggcgcggcgtcgctgggtgcaccgcgaccacgggcagagccacgcggcgggaggactacaactcccggcacaccccgcgccgccccgcctctactcccagaaggccgcggggggtggaccgcctaagagggcgtgcgctcccgacatgccccgcggcgcgccattaaccgccagatttgagtcgcgggacccgttggcagaggtgggaattcaccggtcaccatggttctggggccctgcatgctgctgctgctgctgctgctgggcctgaggctacagctctccctgggcatcatcccagttgaggaagagaacccggacttctggaaccgcgaggcagccgaggccctgggtgccgccaagaagctgcagcctgcacagacagccgccaagaacctcatcatcttcctgggcgatgggatgggggtgtctacggtgacagctgccaggatcctaaaagggcagaagaaggacaaactggggcctgagatacccctggctatggaccgcttcccatatgtggctctgtccaagacatacaatgtagacaaacatgtgccagacagtggagccacagccacggcctacctgtgcggggtcaagggcaacttccagaccattggcttgagtgcagccgcccgctttaaccagtgcaacacgacacgcggcaacgaggtcatctccgtgatgaatcgggccaagaaagcagggaagtcagtgggagtggtaaccaccacacgagtgcagcacgcctcgccagccggcacctacgcccacacggtgaaccgcaactggtactcggacgccgacgtgcctgcctcggcccgccaggaggggtgccaggacatcgctacgcagctcatctccaacatggacattgatgtgatcctgggtggaggccgaaagtacatgtttcgcatgggaaccccagaccctgagtacccagatgactacagccaaggtgggaccaggctggacgggaagaatctggtgcaggaatggctggcgaagcgccagggtgcccggtatgtgtggaaccgcactgagctcatgcaggcttccctggacccgtctgtgacccatctcatgggtctctttgagcctggagacatgaaatacgagatccaccgagactccacactggacccctccctgatggagatgacagaggctgccctgcgcctgctgagcaggaacccccgcggcttcttcctcttcgtggagggtggtcgcatcgaccacggtcatcacgaaagcagggcttaccgggcactgactgagacgatcatgttcgacgacgccattgagagggcgggccagctcaccagcgaggaggacacgctgagcctcgtcactgccgaccactcccacgtcttctccttcggaggctaccccctgcgagggagctccatcttcgggctggcccctggcaaggcccgggacaggaaggcctacacggtcctcctatacggaaacggtccaggctatgtgctcaaggacggcgcccggccggatgttaccgagagcgagagcgggagccccgagtatcggcagcagtcagcagtgcccctggacgaagagacccacgcaggcgaggacgtggcggtgttcgcgcgcggcccgcaggcgcacctggttcacggcgtgcaggagcagaccttcatagcgcacgtcatggccttcgccgcctgcctggagccctacaccgcctgcgacctggcgccccccgccggcaccaccgacgccgcgcacccggggcggtcccggtccaagcgtctggattgagctagcttcgaatttaaatcggatccctgcaggagctcgtcgacaatcaacctctggattacaaaatttgtgaaagattgactggtattcttaactatgttgctccttttacgctatgtggatacgctgctttaatgcctttgtatcatgctattgcttcccgtatggctttcattttctcctccttgtataaatcctggttgctgtctctttatgaggagttgtggcccgttgtcaggcaacgtggcgtggtgtgcactgtgtttgctgacgcaacccccactggttggggcattgccaccacctgtcagctcctttccgggactttcgctttccccctccctattgccacggcggaactcatcgccgcctgccttgcccgctgctggacaggggctcggctgttgggcactgacaattccgtggtgttgtcggggaaatcatcgtcctttccttggctgctcgcctgtgttgccacctggattctgcgcgggacgtccttctgctacgtcccttcggccctcaatccagcggaccttccttcccgcggcctgctgccggctctgcggcctcttccgcgtcttcgccttcgccctcagacgagtcggatctccctttgggccgcctccccgcctggtacaagtaaccgcgaattcctgtgccttctagttgccagccatctgttgtttgcccctcccccgtgccttccttgaccctggaaggtgccactcccactgtcctttcctaataaaatgaggaaattgcatcgcattgtctgagtaggtgtcattctattctggggggtggggtggggcaggacagcaagggggaggattgggaagacaatagcaggcatgctggggatgcggtgggctctatggcccgggacggccgctagcccgcctaatgagcgggcttttttttggcttgttgtccacaaccgttaaaccttaaaagctttaaaagccttatatattcttttttttcttataaaacttaaaaccttagaggctatttaagttgctgatttatattaattttattgttcaaacatgagagcttagtacgtgaaacatgagagcttagtacgttagccatgagagcttagtacgttagccatgagggtttagttcgttaaacatgagagcttagtacgttaaacatgagagcttagtacgtactatcaacaggttgaactgctgatccacgttgtggtagaattggtaaagagagtcgtgtaaaatatcgagttcgcacatcttgttgtctgattattgatttttggcgaaaccatttgatcatatgacaagatgtgtatctaccttaacttaatgattttgataaaaatcattaggtacggccgcggtgccagggcgtgcccttgggctccccgggcgcgactagt

SEQ ID NO: 6 - RNA, 21 nt, synthetic construct
  misc_feature 1..21: note = Description of Artificial Sequence: Synthetic oligonucleotide
  source 1..21: mol_type = other RNA
aaatgtactgcgcgtggagac

SEQ ID NO: 7 - protein, 8 aa, synthetic construct
  REGION 1..8: note = Description of Artificial Sequence: Synthetic peptide
DYKDDDDK